European Patent Application EP 4 722 231 A1, published April 8, 2026. Title: 一种广谱抗病毒多肽的生物合成方法. Applicant: 山西锦波生物医药股份有限公司. Application CN. The sequence listing filed with the application follows.

SEQUENCE LISTING (2 sequences)

SEQ ID NO: 1 - protein, 36 aa, synthetic construct
SLDQINVTFLDLEYEMKKLEEAIKKLEESYIDLKEL

SEQ ID NO: 2 - DNA, 108 bp, synthetic construct
  source 1..108: mol_type = other DNA
agcctggatcagattaatgtgacctttctggatctggaatatgaaatgaaaaagctggaagaagccattaagaaactggaagaaagttatattgacctgaaagaactg